European Patent Specification EP 3 955 921 B1, published August 12, 2026. Title: HIV PROTEASE INHIBITORS. Applicant: Gilead Sciences, Inc. The sequence listing filed with the application follows.

SEQUENCE LISTING (1 sequence)

SEQ ID NO: 1 - protein, 6 aa, Artificial Sequence
  synthetic polypeptide substrate
  MOD_RES (1)..(1): 2-aminobenzoyl
  misc_feature (3)..(3): Xaa = norleucine (Nle)
  MOD_RES (4)..(4): p-nitro
TIXFQR